European Patent Specification EP 3 958 831 B1, published February 26, 2025. Title: Prebiotic skin care compositions containing carboxylic acids. Applicant: Universiteit Gent. The sequence listing filed with the application follows.

SEQUENCE LISTING (9 sequences)

SEQ ID NO: 1 - DNA, 1111 bp, Staphylococcus epidermidis
tcctctgacgttagcggcggacgggtgagtaacacgtggataacctacctataagactgggataacttcgggaaaccggagctaataccggataatatattgaaccgcatggttcaatagtgaaagacggttttgctgtcacttatagatggatccgcgccgcattagctagttggtaaggtaacggcttaccaaggcaacgatgcgtagccgacctgagagggtgatcggccacactggaactgagacacggtccagactcctacgggaggcagcagtagggaatcttccgcaatgggcgaaagcctgacggagcaacgccgcgtgagtgatgaaggtcttcggatcgtaaaactctgttattagggaagaacaaatgtgtaagtaactatgcacgtcttgacggtacctaatcagaaagccacggctaactacgtgccagcagccgcggtaatacgtaggtggcaagcgttatccggaattattgggcgtaaagcgcgcgtaggcggttttttaagtctgatgtgaaagcccacggctcaaccgtggagggtcattggaaactggaaaacttgagtgcagaagaggaaagtggaattccatgtgtagcggtgaaatgcgcagagatatggaggaacaccagtggcgaaggcgactttctggtctgtaactgacgctgatgtgcgaaagcgtggggatcaaacaggattagataccctggtagtccacgccgtaaacgatgagtgctaagtgttagggggtttccgccccttagtgctgcagctaacgcattaagcactccgcctggggagtacgaccgcaaggttgaaactcaaaggaattgacggggacccgcacaagcggtggagcatgtggtttaattcgaagcaacgcgaagaaccttaccaaatcttgacatcctctgacccctctagagatagagttttccccttcgggggacagagtgacaggtggtgcatggttgtcgtcagctcgtgtcgtgagatgttgggttaagtcccgcaacgagcgcaacccttaagcttagttgccatcattaagttgggcactctaagttgactgccggtgacaaaccggaagaaaggtgggg

SEQ ID NO: 2 - DNA, 1000 bp, Acinetobacter lwoffii
tggggtaaaggcctaccaaggcgacgatctgtagcgggtctgagaggatgatccgccacactgggactgagacacggcccagactcctacgggaggcagcagtggggaatattggacaatggggggaaccctgatccagccatgccgcgtgtgtgaagaaggccttttggttgtaaagcactttaagcgaggaggaggctaccgagattaatactcttggatagtggacgttactcgcagaataagcaccggctaactctgtgccagcagccgcggtaatacagagggtgcaagcgttaatcggatttactgggcgtaaagcgcgcgtaggtggccaattaagtcaaatgtgaaatccccgagcttaacttgggaattgcattcgatactggttggctagagtatgggagaggatggtagaattccaggtgtagcggtgaaatgcgtagagatctggaggaataccgatggcgaaggcagccatctggcctaatactgacactgaggtgcgaaagcatggggagcaaacaggattagataccctggtagtccatgccgtaaacgatgtctactagccgttggggcctttgaggctttagtggcgcagctaacgcgataagtagaccgcctggggagtacggtcgcaagactaaaactcaaatgaattgacgggggcccgcacaagcggtggagcatgtggtttaattcgatgcaacgcgaagaaccttacctggtcttgacatagtaagaactttccagagatggattggtgccttcgggaacttacatacaggtgctgcatggctgtcgtcagctcgtgtcgtgagatgttgggttaagtcccgcaacgagcgcaacccttttccttatttgccagcgggttaagccgggaactttaaggatactgccagtgacaaactggaggaaggcggggacgacgtcaagtcatcatggcccttacgaccagggctacacacgtgctacaatggtcggtacaaag

SEQ ID NO: 3 - DNA, 848 bp, Propionibacterium acnes (Cutibacterium acnes)
ggtagccggcctgagagggtgaccggccacattgggactgagatacggcccagactcctacgggaggcagcagtggggaatattgcacaatgggcggaagcctgatgcagcaacgccgcgtgcgggatgacggccttcgggttgtaaaccgctttcgcctgtgaccaagcgtgagtgacggtaatgggtaaagaagcaccggctaactacgtgccagcagccgcggtgatacgcagggtgcgagcgttgtccggatttattgggcgtaaagggctcgtaggtggttgatcgcgtcggaagtgtaatcttggggcttaaccctgagcgtgctttcgatacgggttgacttgaggaaggtaggggagaatggaattcctggtggagcggtggaatgcgcagatatcaggaggaacaccagtggcgaaggcggttctctgggcctttcctgacgctgaggagcgaaagcgtggggagcgaacaggcttagataccctggtagtccacgctgtaaacggtgggtactaggcgtggggtccattccaccgggttccgtggccgtagctaacgcttcaagtaccccgcctggggagtacggccgcaaggctaaaactcaaaggaattgacggggccccgcacaagcggcggagcatgcggattaattagatgccacgcctagaaccttacctgggcttgacacggatcgggagtgctcagagatgggtgtgcgctcttttggggtcggttcacaggcggtgcatggctgtcgtcagctcgtgtcgtgagatgttgggataagtcccgcaacgagcgcaacccttcttccctgctgccagcacgttatggcgggg

SEQ ID NO: 4 - DNA, 795 bp, Enhydrobacter aerosaccus
ccggactcctacgggaggcagcagtggggaatattggacaatgggggcaaccctgatccagccatgccgcgtgtgtgaagaaggccttttggttgtaaagcactttaagcagggaggagaggctaatggttaatacccattagattagacgttacctgcagaataagcaccggctaactctgtgccagcagccgcggtaatacagagggtgcgagcgttaatcggaattactgggcgtaaagcgagtgtaggtggctcattaagtcacatgtgaaatccccgggcttaacctgggaactgcatgtgatactggtggtgctagaatatgtgagagggaagtagaattccaggtgtagcggtgaaatgcgtagagatctggaggaataccgatggcgaaggcagcttcctggcataatattgacactgagattcgaaagcgtgggtagcaaacaggattagataccctggtagtccacgccgtaaacgatgtctactagccgttggggtccttgagactttagtggcgcagttaacgcgataagtagaccgcctggggagtacggccgcaaggttaaaactcaaatgaattgacgggggcccgcacaagcggtggagcatgtggtttaattcgatgcaacgcgaagaaccttacctggtgctatgactcatagctgagaatgctgctgcagagatgagagagtgccttcgggaactcacatacaggtgctgcatggctgtcgtcagctcgtgtcgtgagatgttgggttaagtcccgcaacgagcgcaacccttttc

SEQ ID NO: 5 - DNA, 642 bp, Corynebacterium tuberculostearicum
cgggtgagtaacacgtgggtgatctgccctgcacttcgggataagcctgggaaactgggtctaataccggataggagccatttttagtgtgatggttggaaagttttttcggtgtaggatgagctcgcggcctatcagcttgttggtggggtaatggcctaccaaggcggcgacgggtagccggcctgagagggtggacggccacattgggactgagatacggcccagactcctacgggaggcagcagtggggaatattgcacaatgggcgcaagcctgatgcagcgacgccgcgtgggggatgacggccttcgggttgtaaactcctttcgctagggacgaagctttttgtgacggtacctagataaaaagcaccggctaactacgtgccagcagccgcggtaatacgtagggtgcgagcgttgtccggaattactgggcgtaaagggctcgtaggtggtttgtcgcgtcgtctgtgaaattccggggcttaactccgggcgtgcaggcgatacggccataacttgagtactgtaggggtaactggaattcctggggtagcgctgaaatgcgcagatatcaggaggaacaccgatggcgaaggcaggttactgggcagttactgacgctgagaagcgaaag

SEQ ID NO: 6 - DNA, 1054 bp, Corynebacterium amycolatum
gtggcgaacgggtgagtaacacgtgggtgacctgccctgcacttcgggataagcctgggaaactgggtctaataccggataggaccgcaccgtgagggtgtggtggaaagttttttcggtgtgggatgggcccgcggcctatcagcttgttggtggggtaatggcctaccaaggcggcgacgggtagccggcctgagagggtggacggccacattgggactgagacacggcccagactcctacgggaggcagcagtggggaatattgcacaatgggcggaagcctgatgcagcgacgccgcgtgggggatgacggccttcgggttgtaaactcctttcaccatcgacgaagggtttctgacggtagatggagaagaagcaccggctaactacgtgccagcagccgcggtaatacgtagggtgcgagcgttgtccggaattactgggcgtaaagagctcgtaggtggtttgtcgcgtcgtctgtgaaattccggggcttaactccgggcgtgcaggcgatacgggcataacttgagtactgtaggggagactggaattcctggtgtagcggtgaaatgcgcagatatcaggaggaacaccggtggcgaaggcgggtctctgggcagtaactgacgctgaggagcgaaagcatggggagcgaacaggattagataccctggtagtccatgccgtaaacggtgggcgctaggtgtgggtttccttccacgggatccgtgccgtagctaacgcattaagcgccccgcctggggagtacggccgcaaggctaaaactcaaaggaattgacgggggcccgcacaagcggcggagcatgtggattaattcgatgcaacgcgaagaaccttacctgggcttgacatatacaggatcgcgccagagatggtgtttcccttgtggcttgtatacaggtggtgcatggttgtcgtcagctcgtgtcgtgagatgttgggttaagtcccgcaacgagcgcaacccttgtcttatgttgccagcacgttgtggtgggggactcgtaaagaaactgcccggggttaac

SEQ ID NO: 7 - DNA, 1082 bp, Staphylococcus hominis
gttagcggcggacgggtgagtaacacgtaggtaacctacctataagactgggataacttcgggaaaccggagctaataccggataatatttcgaaccgcatggttcgatagtgaaagatggctttgctatcacttatagatggacctgcgccgtattagctagttggtaaggtaacggcttaccaaggcaacgatacgtagccgacctgagagggtgatcggccacactggaactgagacacggtccagactcctacgggaggcagcagtagggaatcttccgcaatgggcgaaagcctgacggagcaacgccgcgtgagtgatgaaggtcttcggatcgtaaaactctgttattagggaagaacaaacgtgtaagtaactgtgcacgtcttgacggtacctaatcagaaagccacggctaactacgtgccagcagccgcggtaatacgtaggtggcaagcgttatccggaattattgggcgtaaagcgcgcgtaggcggttttttaagtctgatgtgaaagcccacggctcaaccgtggagggtcattggaaactggaaaacttgagtgcagaagaggaaagtggaattcctggtgtagcggtgaaatgcgcagagatatggaggaacaccagtggcgaaggcgactttctggtctgtaactgacgctgatgtgcgaaagcgtggggatcaaacaggattagataccctggtagtccacgccgtaaacgatgagtgctaagtgttaagggggtttccgccccttagtgctgcagctaacgcattaagcactccgcctggggagtacgaccgcaaggttgaaactcaaaggaattgacggggacccgcacaagcggtggagcatgtggtttaattcgaagcaacgcgaagaaccttaccaaatcttgacatcctttgacccttctagaagatagaagtttccccttcgggggacaaagtgacaggtggtgcatggttgtcgtcagctcgtgtcgtgagatgtttgggttaagtcccgcaacgagcgcaacccttaagcttagttgccatcattaagttgggcactctaagttgactgccggt

SEQ ID NO: 8 - DNA, 579 bp, Enterobacter cloacae
gagtggcggacgggtgagtaatgtctgggaaactgcctgatggagggggataactactggaaacggtagctaataccgcataatgtcgcaagaccaaagagggggaccttcgggcctcttgccatcagatgtgcccagatgggattagctagtaggtggggtaacggctcacctaggcgacgatccctagctggtctgagaggatgaccagccacactggaactgagacacggtccagactcctacgggaggcagcagtggggaatattgcacaatgggcgcaagcctgatgcagccatgccgcgtgtatgaagaaggccttcgggttgtaaagtactttcagcggggaggaaggtgttgtggttaataaccgcagcaattgacgttacccgcagaagaagcaccggctaactccgtgccagcagccgcggtaatacggagggtgcaagcgttaatcggaattactgggcgtaaagcgcacgcaggcggtctgtcaagtcggatgtgaaatccccgggctcaacctgggaactgcattcgaaactggcaggctggagtcttgtagaggggggtagaatt

SEQ ID NO: 9 - DNA, 887 bp, Micrococcus luteus
gggtgagtaacacgtgagtaacctgcccttaactctgggataagcctgggaaactgggtctaataccggataggagcgcccaccgcatggtgggtgttggaaagatttatcggttttggatggactcgcggcctatcagcttgttggtgaggtaatggctcaccaaggcgacgacgggtagccggcctgagagggtgaccggccacactgggactgagacacggcccagactcctacgggaggcagcagtggggaatattgcacaatgggcgaaagcctgatgcagcgacgccgcgtgagggatgacggccttcgggttgtaaacctctttcagtagggaagaagcgaaagtgacggtacctgcagaagaagcaccggctaactacgtgccagcagccgcggtaatacgtagggtgcgagcgttatccggaattattgggcgtaaagagctcgtaggcggtttgtcgcgtctgtcgtgaaagtccggggcttaaccccggatctgcggtgggtacgggcagactagagtgcagtaggggagactggaattcctggtgtagcggtggaatgcgcagatatcaggaggaacaccgatggcgaaggcaggtctctgggctgtaactgacgctgaggagcgaaagcatggggagcgaacaggattagataccctggtagtccatgccgtaaacgttgggcactaggtgtggggaccattccacggtttccgcgccgcagctaacgcattaagtgccccgcctggggagtacggccgcaaggctaaaactcaaaggaattgacgggggcccgcacaagcggcggagcatgcggattaattcgatgcaacgcgaaagaaccttaccaaggcttgacatgttctcgatcgccgt